European Patent Specification EP 3 565 837 B1, published April 10, 2024. Title: COMBINED TREATMENT WITH NETRIN-1 INTERFERING DRUG AND IMMUNE CHECKPOINT INHIBITORS DRUGS. Applicant: NETRIS PHARMA. The sequence listing filed with the application follows.

SEQUENCE LISTING (36 sequences)

SEQ ID NO: 1 - protein, 604 aa, Homo sapiens
  SIGNAL (1)..(24)
  MISC_FEATURE (339)..(381): linear epitope
MMRAVWEALAALAAVACLVGAVRGGPGLSMFAGQAAQPDPCSDENGHPRRCIPDFVNAAFGKDVRVSSTCGRPPARYCVVSERGEERLRSCHLCNASDPKKAHPPAFLTDLNNPHNLTCWQSENYLQFPHNVTLTLSLGKKFEVTYVSLQFCSPRPESMAIYKSMDYGRTWVPFQFYSTQCRKMYNRPHRAPITKQNEQEAVCTDSHTDMRPLSGGLIAFSTLDGRPSAHDFDNSPVLQDWVTATDIRVAFSRLHTFGDENEDDSELARDSYFYAVSDLQVGGRCKCNGHAARCVRDRDDSLVCDCRHNTAGPECDRCKPFHYDRPWQRATAREANECVACNCNLHARRCRFNMELYKLSGRKSGGVCLNCRHNTAGRHCHYCKEGYYRDMGKPITHRKACKACDCHPVGAAGKTCNQTTGQCPCKDGVTGITCNRCAKGYQQSRSPIAPCIKIPVAPPTTAASSVEEPEDCDSYCKASKGKLKINMKKYCKKDYAVQIHILKADKAGDWWKFTVNIISVYKQGTSRIRRGDQSLWIRSRDIACKCPKIKPLKKYLLLGNAEDSPDQSGIVADKSSLVIQWRDTWARRLRKFQQREKKGKCKKA

SEQ ID NO: 2 - DNA, 1817 bp, Homo sapiens
atgatgcgcgcagtgtgggaggcgctggcggcgctggcggcggtggcgtgcctggtgggcgcggtgcgcggcgggcccgggctcagcatgttcgcgggccaggcggcgcagcccgatccctgctcggacgagaacggccacccgcgccgctgcatcccggactttgtcaatgcggccttcggcaaggacgtgcgcgtgtccagcacctgcggccggcccccggcgcgctactgcgtggtgagcgagcgcggcgaggagcggctgcgctcgtgccacctctgcaacgcgtccgaccccaagaaggcgcacccgcccgccttcctcaccgacctcaacaacccgcacaacctgacgtgctggcagtccgagaactacctgcagttcccgcacaacgtcacgctcacactgtccctcggcaagaagttcgaagtgacctacgtgagcctgcagttctgctcgccgcggcccgagtccatggccatctacaagtccatggactacgggcgcacgtgggtgcccttccagttctactccacgcagtgccgcaagatgtacaaccggccgcaccgcgcgcccatcaccaagcagaacgagcaggaggccgtgtgcaccgactcgcacaccgacatgcgcccgctctcgggcggcctcatcgccttcagcacgctggacgggcggccctcggcgcacgacttcgacaactcgcccgtgctgcaggactgggtcacggccacagacatccgcgtggccttcagccgcctgcacacgttcggcgacgagaacgaggacgactcggagctggcgcgcgactcgtacttctacgcggtgtccgacctgcaggtgggcggccggtgcaagtgcaacggccacgcggcccgctgcgtgcgcgaccgcgacgacagcctggtgtgcgactgcaggcacaacacggccggcccggagtgcgaccgctgcaagcccttccactacgaccggccctggcagcgcgccacagcccgcgaagccaacgagtgcgtggcctgtaactgcaacctgcatgcccggcgctgccgcttcaacatggagctctacaagctttcggggcgcaagagcggaggtgtctgcctcaactgtcgccacaacaccgccggccgccactgccattactgcaaggagggctactaccgcgacatgggcaagcccatcacccaccggaaggcctgcaaagcctgtgattgccaccctgtgggtgctgctggcaaaacctgcaaccaaaccaccggccagtgtccctgcaaggacggcgtgacgggtatcacctgcaaccgctgcgccaaaggctaccagcagagccgctctcccatcgccccctgcataaagatccctgtagcgccgccgacgactgcagccagcagcgtggaggagcctgaagactgcgattcctactgcaaggcctccaaggggaagctgaagattaacatgaaaaagtactgcaagaaggactatgccgtccagatccacatcctgaaggcggacaaggcgggggactggtggaagttcacggtgaacatcatctccgtgtataagcagggcacgagccgcatccgccgcggtgaccagagcctgtggatccgctcgcgggacatcgcctgcaagtgtcccaaaatcaagcccctcaagaagtacctgctgctgggcaacgcggaggactctccggaccagagcggcatcgtggccgataaaagcagcctggtgatccagtggcgggacacgtgggcgcggcggctgcgcaagttccagcagcgtgagaagaagggcaagtgcaagaaggcctagcg

SEQ ID NO: 3 - protein, 43 aa, Homo sapiens
VACNCNLHARRCRFNMELYKLSGRKSGGVCLNCRHNTAGRHCH

SEQ ID NO: 4 - DNA, 129 bp, Homo sapiens
gtggcctgtaactgcaacctgcatgcccggcgctgccgcttcaacatggagctctacaagctttcggggcgcaagagcggaggtgtctgcctcaactgtcgccacaacaccgccggccgccactgccat

SEQ ID NO: 5 - protein, 8 aa, Mus musculus
GYTFTSYN

SEQ ID NO: 6 - protein, 8 aa, Mus musculus
IYPGNGDT

SEQ ID NO: 7 - protein, 9 aa, Mus musculus
ARGGTGFAY

SEQ ID NO: 8 - protein, 6 aa, Mus musculus
QSVSND

SEQ ID NO: 9 - protein, 9 aa, Mus musculus
QQDYSSPWT

SEQ ID NO: 10 - protein, 116 aa, Mus musculus
  MISC_FEATURE (26)..(33): CDR according to IGMT
  MISC_FEATURE (51)..(58): CDR according to IGMT
  MISC_FEATURE (97)..(105): CDR according to IGMT
QAYLQQSGAELVRPGASVKMSCKASGYTFTSYNMHWVKQTPRQGLEWIGAIYPGNGDTSYNQKFKGKATLTVDKSSSTAYMQLSSLTSEDSAVYFCARGGTGFAYWGQGTLVTVSA

SEQ ID NO: 11 - protein, 107 aa, Mus musculus
  MISC_FEATURE (27)..(32): CDR according to IGMT
  MISC_FEATURE (50)..(52): CDR according to IGMT
  MISC_FEATURE (89)..(97): CDR according to IGMT
SIVMTQTPKFLLVSAGDRVTITCKASQSVSNDVAWYQQKPGQSPKLLIYYASNRYTGVPDRFTGSGYGTDFTFTISTVQAEDLAVYFCQQDYSSPWTFGGGTKLEIK

SEQ ID NO: 12 - protein, 440 aa, Mus musculus
  MISC_FEATURE (26)..(33): CDR according to IGMT
  MISC_FEATURE (51)..(58): CDR according to IGMT
  MISC_FEATURE (97)..(105): CDR according to IGMT
QAYLQQSGAELVRPGASVKMSCKASGYTFTSYNMHWVKQTPRQGLEWIGAIYPGNGDTSYNQKFKGKATLTVDKSSSTAYMQLSSLTSEDSAVYFCARGGTGFAYWGQGTLVTVSAAKTTPPSVYPLAPGSAAQTNSMVTLGCLVKGYFPEPVTVTWNSGSLSSGVHTFPAVLESDLYTLSSSVTVPSSPRPSETVTCNVAHPASSTKVDKKIVPRDCGCKPCICTVPEVSSVFIFPPKPKDVLTITLTPKVTCVVVDISKDDPEVQFSWFVDDVEVHTAQTQPREEQFNSTFRSVSELPIMHQDWLNGKEFKCRVNSAAFPAPIEKTISKTKGRPKAPQVYTIPPPKEQMAKDKVSLTCMITDFFPEDITVEWQWNGQPAENYKNTQPIMNTNGSYFVYSKLNVQKSNWEAGNTFTCSVLHEGLHNHHTEKSLSHSPGK

SEQ ID NO: 13 - protein, 214 aa, Mus musculus
  MISC_FEATURE (27)..(32): CDR according to IGMT
  MISC_FEATURE (50)..(52): CDR according to IGMT
  MISC_FEATURE (89)..(97): CDR according to IGMT
SIVMTQTPKFLLVSAGDRVTITCKASQSVSNDVAWYQQKPGQSPKLLIYYASNRYTGVPDRFTGSGYGTDFTFTISTVQAEDLAVYFCQQDYSSPWTFGGGTKLEIKRADAAPTVSIFPPSSEQLTSGGASVVCFLNNFYPKDINVKWKIDGSERQNGVLNSWTDQDSKDSTYSMSSTLTLTKDEYERHNSYTCEATHKTSTSPIVKSFNRNEC

SEQ ID NO: 14 - protein, 101 aa, Artificial Sequence
  humanized variant
  MISC_FEATURE (27)..(32): CDR according to IGMT
  MISC_FEATURE (50)..(52): CDR according to IGMT
  MISC_FEATURE (89)..(97): CDR according to IGMT
EIVMTQSPATLSVSPGERATLSCKASQSVSNDVAWYQQKPGKAPKLLIYYASNRYTGIPPRFSGSGYGTDFTLTINNIESEDAAYYFCQQDYSSPWTFGQG

SEQ ID NO: 15 - protein, 101 aa, Artificial Sequence
  humanized variant
  MISC_FEATURE (27)..(32): CDR according to IGMT
  MISC_FEATURE (50)..(52): CDR according to IGMT
  MISC_FEATURE (89)..(97): CDR according to IGMT
DIQMTQSPSSLSASVGDRVTITCKASQSVSNDVAWFQQRPGQSPRRLIYYASNRYTGVPSRFSGSGSGTDFTFTISSLEAEDAATYYCQQDYSSPWTFGQG

SEQ ID NO: 16 - protein, 101 aa, Artificial Sequence
  humanized variant
  MISC_FEATURE (27)..(32): CDR according to IGMT
  MISC_FEATURE (50)..(52): CDR according to IGMT
  MISC_FEATURE (89)..(97): CDR according to IGMT
DIQMTQSPSSLSASVGDRVTITCKASQSVSNDVAWYQQKPGQAPRLLIYYASNRYTGIPPRFSGSGYGTDFTLTINNIESEDAAYYFCQQDYSSPWTFGQG

SEQ ID NO: 17 - protein, 101 aa, Artificial Sequence
  humanized variant
  MISC_FEATURE (27)..(32): CDR according to IGMT
  MISC_FEATURE (50)..(52): CDR according to IGMT
  MISC_FEATURE (89)..(97): CDR according to IGMT
DIQMTQSPSSLSASVGDRVTITCKASQSVSNDVAWYLQKPGQSPQLLIYYASNRYTGVPSRFSGSGSGTDFTFTISSLEAEDAATYYCQQDYSSPWTFGQG

SEQ ID NO: 18 - protein, 101 aa, Artificial Sequence
  humanized variant
  MISC_FEATURE (27)..(32): CDR according to IGMT
  MISC_FEATURE (50)..(52): CDR according to IGMT
  MISC_FEATURE (89)..(97): CDR according to IGMT
DIVMTQTPLSLPVTPGEPASISCKASQSVSNDVAWYQQKPGQAPRLLIYYASNRYTGIPPRFSGSGYGTDFTLTINNIESEDAAYYFCQQDYSSPWTFGQG

SEQ ID NO: 19 - protein, 101 aa, Artificial Sequence
  humanized variant
  MISC_FEATURE (27)..(32): CDR according to IGMT
  MISC_FEATURE (50)..(52): CDR according to IGMT
  MISC_FEATURE (89)..(97): CDR according to IGMT
EIVMTQSPATLSVSPGERATLSCRASQSVSNDVAWYQQKPGQAPRLLIYYASNRYTGIPARFSGSGSGTEFTLTISSLQSEDFAVYYCQQDYSSPWTFGQG

SEQ ID NO: 20 - protein, 109 aa, Artificial Sequence
  humanized variant
  MISC_FEATURE (26)..(33): CDR according to IGMT
  MISC_FEATURE (51)..(58): CDR according to IGMT
  MISC_FEATURE (97)..(105): CDR according to IGMT
QVQLVQSGAEVKKPGASVKVSCKASGYTFTSYNMHWVRQATGQGLEWMGAIYPGNGDTSYNQKFKGRVTITADKSTSTAYMELSSLRSEDTAVYYCARGGTGFAYWGQG

SEQ ID NO: 21 - protein, 109 aa, Artificial Sequence
  humanized variant
  MISC_FEATURE (26)..(33): CDR according to IGMT
  MISC_FEATURE (51)..(58): CDR according to IGMT
  MISC_FEATURE (97)..(105): CDR according to IGMT
QVQLQQSGPGLVKPSQTLSLTCAISGYTFTSYNMHWIRQPPGKGLEWIGAIYPGNGDTSYNQKFKGRVTITADKSTSTAYMELSSLRSEDTAVYYCARGGTGFAYWGQG

SEQ ID NO: 22 - protein, 109 aa, Artificial Sequence
  humanized variant
  MISC_FEATURE (26)..(33): CDR according to IGMT
  MISC_FEATURE (51)..(58): CDR according to IGMT
  MISC_FEATURE (97)..(105): CDR according to IGMT
QVQLQQSGPGLVKPSQTLSLTCAISGYTFTSYNMHWVRQATGQGLEWMGAIYPGNGDTSYNQKFKGRLTISKDTSKNQVVLTMTNMDPVDTATYYCARGGTGFAYWGQG

SEQ ID NO: 23 - protein, 109 aa, Artificial Sequence
  humanized variant
  MISC_FEATURE (26)..(33): CDR according to IGMT
  MISC_FEATURE (51)..(58): CDR according to IGMT
  MISC_FEATURE (97)..(105): CDR according to IGMT
EVQLVQSGAEVKKPGESLRISCKGSGYTFTSYNMHWVRQATGQGLEWMGAIYPGNGDTSYNQKFKGRFTISRDDSKNTAYLQMNSLKTEDTAVYYCARGGTGFAYWGQG

SEQ ID NO: 24 - protein, 109 aa, Artificial Sequence
  humanized variant
  MISC_FEATURE (26)..(33): CDR according to IGMT
  MISC_FEATURE (51)..(58): CDR according to IGMT
  MISC_FEATURE (97)..(105): CDR according to IGMT
QVQLQESGPGLVKPSQTLSLTCTVSGYTFTSYNMHWVRQAPGQGLEWMGAIYPGNGDTSYNQKFKGRVTISVDTSKNQFSLKLSSVTAADTAVYYCARGGTGFAYWGQG

SEQ ID NO: 25 - protein, 109 aa, Artificial Sequence; identical to SEQ ID NO: 20
  humanized variant
  MISC_FEATURE (26)..(33): CDR according to IGMT
  MISC_FEATURE (51)..(58): CDR according to IGMT
  MISC_FEATURE (97)..(105): CDR according to IGMT

SEQ ID NO: 26 - protein, 109 aa, Artificial Sequence
  humanized variant
  MISC_FEATURE (26)..(33): CDR according to IGMT
  MISC_FEATURE (51)..(58): CDR according to IGMT
  MISC_FEATURE (97)..(105): CDR according to IGMT
QVQLQQSGPGLVKPSQTLSLTCAISGYTFTSYNMHWVRQATGQGLEWMGAIYPGNGDTSYNQKFKGRVTITADKSTSTAYMELSSLRSEDTAVYYCARGGTGFAYWGQG

SEQ ID NO: 27 - protein, 108 aa, Artificial Sequence
  humanized variant
  MISC_FEATURE (26)..(33): CDR according to IGMT
  MISC_FEATURE (51)..(58): CDR according to IGMT
  MISC_FEATURE (97)..(105): CDR according to IGMT
QVQLVQSGAEVKKPGASVKVSCKASGYTFTSYNMHWVRQAPGQGLEWMGAIYPGNGDTSYAQKFKGRVTMTRDTSTSTVYMELSSLRSEDTAVYYCARGGTGFAYWGQ

SEQ ID NO: 28 - protein, 5 aa, Mus musculus
SYNMH

SEQ ID NO: 29 - protein, 17 aa, Mus musculus
AIYPGNGDTSYNQKFKG

SEQ ID NO: 30 - protein, 7 aa, Mus musculus
GGTGFAY

SEQ ID NO: 31 - protein, 11 aa, Mus musculus
KASQSVSNDVA

SEQ ID NO: 32 - protein, 7 aa, Mus musculus
YASNRYT

SEQ ID NO: 33 - DNA, 25 bp, Artificial Sequence
  forward primer for PCR of human netrin-1 gene
aaaagtactgcaagaaggactatgc

SEQ ID NO: 34 - DNA, 21 bp, Artificial Sequence
  reverse primer for PCR of human netrin-1 gene
ccctgcttatacacggagatg

SEQ ID NO: 35 - protein, 22 aa, Homo sapiens
ARRCRFNMELYKLSGRKSGGVC

SEQ ID NO: 36 - DNA, 66 bp, cDNA
gcccggcgctgccgcttcaacatggagctctacaagctttcggggcgcaagagcggaggtgtctgc